European Patent Specification EP 3 911 330 B1, published March 5, 2025. Title: Small molecules for increasing precise genome editing efficiency. Applicant: Max-Planck-Gesellschaft zur Förderung der Wissenschaften e.V. The sequence listing filed with the application follows.

SEQUENCE LISTING (63 sequences)

SEQ ID NO: 1 - DNA, 20 bp, Artificial Sequence
  gRNA LYPLA1 t1
tgaacgtggctatgccttca

SEQ ID NO: 2 - DNA, 20 bp, Artificial Sequence
  gRNA LYPLA1 t2
acaggcctaacaggcctaca

SEQ ID NO: 3 - DNA, 20 bp, Artificial Sequence
  gRNA SCAP1 t1
ctctgggatcaggagcttgg

SEQ ID NO: 4 - DNA, 20 bp, Artificial Sequence
  gRNA SCAP t2
gctgcacaggagacaggaca

SEQ ID NO: 5 - DNA, 20 bp, Artificial Sequence
  gRNA SSH2 t1
cagatcctcaggagggccca

SEQ ID NO: 6 - DNA, 20 bp, Artificial Sequence
  gRNA SSH2 t2
gtggtcaaactccagcacct

SEQ ID NO: 7 - DNA, 20 bp, Artificial Sequence
  gRNA CSGALNACT1 t1
ctcatcttatttcgaccatt

SEQ ID NO: 8 - DNA, 20 bp, Artificial Sequence
  gRNA CSGALNACT1 t2
gccgtttgaattcgtgtttg

SEQ ID NO: 9 - DNA, 20 bp, Artificial Sequence
  gRNA VCAN t1
gtttactgttgcctgatcat

SEQ ID NO: 10 - DNA, 20 bp, Artificial Sequence
  gRNA VCAN t2
ccctgtggaatttaatactg

SEQ ID NO: 11 - DNA, 20 bp, Artificial Sequence
  gRNA ITGB4 t1
gggtcctggggtgggcagat

SEQ ID NO: 12 - DNA, 20 bp, Artificial Sequence
  gRNA ITGB4 t2
ccgcagctgggcagccgtgc

SEQ ID NO: 13 - DNA, 20 bp, Artificial Sequence
  gRNA FRMD7 t1
agccagctgaaagaagccca

SEQ ID NO: 14 - DNA, 20 bp, Artificial Sequence
  gRNA FRMD7 t2 (also Cas9)
gtgggctctacatagctatg

SEQ ID NO: 15 - DNA, 20 bp, Artificial Sequence
  gRNA PRKDC t1
ggtcctcgccacccttcacc

SEQ ID NO: 16 - DNA, 20 bp, Artificial Sequence
  gRNA PRKDC t2
gcgcgtggagcagctcttcc

SEQ ID NO: 17 - DNA, 20 bp, Artificial Sequence
  gRNA POLQ t1
tagttgaaatgggagtgcaa

SEQ ID NO: 18 - DNA, 20 bp, Artificial Sequence
  gRNA POLQ t2
gtcctgctgcagaatcattc

SEQ ID NO: 19 - DNA, 101 bp, Artificial Sequence
  ssODNs SCAP Cas9n
cttcctaaggcctggcagcaggtcggtcacttgcagacacaactcctccaaggacctggtcccagagctgcacaggagacaggacaaggcacctgctgtgt

SEQ ID NO: 20 - DNA, 113 bp, Artificial Sequence
  ssODNs LYPLA1 Cas9n
ataagtaatataatgttcttattcaataagtaaattcttacttaccatgatggcatagccatgttcatatttaatgtaacaggcctaacaggcctacatggaaaagaaaaaac

SEQ ID NO: 21 - DNA, 106 bp, Artificial Sequence
  ssODNs SSH2 Cas9n
atctgaccctgggccctcctgaggatctggcaagtggtcaaactccagcaccttgggagctggaacagtggcattctgctcagaatgggacagtgagccagcctca

SEQ ID NO: 22 - DNA, 113 bp, Artificial Sequence
  ssODNs CSGALNACT1 Cas9n
gttggccatgttgagcttttcatttttcactttcatgatggggccgaatggacgaaataagacgagccgtttgaattcgtgtttgtggtcccctttgaaggtgagctcataca

SEQ ID NO: 23 - DNA, 101 bp, Artificial Sequence
  ssODNs VCAN Cas9n
gatagcagcatcagaacagcaagtggcagcgagaattcttgattccaataatcaggcaacagtaaaccctgtggaatttaatactgaggttgcaacaccac

SEQ ID NO: 24 - DNA, 105 bp, Artificial Sequence
  ssODNs ITGB4 Cas9n
tggtgatgctgctgtactcgctttgcagcgggtgctggaagagcccggcatggctgcccagctgcgggaagggtcctggggtgggcagataggccagtcagaggg

SEQ ID NO: 25 - DNA, 127 bp, Artificial Sequence
  ssODNs ITGB4 Cas9
ctcacccactaggaagggctcggtggcgctggtgtgggtggtggtgatgctgctgtactcgctttgcagcgggtgctggaagagcccggcatggctgcccagctgcgggaagggtcctggggtgggc

SEQ ID NO: 26 - DNA, 110 bp, Artificial Sequence
  ssODNs FRMD7 Cas9n
aggtgcccagatggtccccaattagagcagaggaaaggacaagtccagatagctatgtagagcccactgcaatgaagccagctgaaagaagcccaaggaatatcagaatg

SEQ ID NO: 27 - DNA, 127 bp, Artificial Sequence
  ssODNs FRMD7 Cas9
tatgcctccccaggtctttttttatgtggacaagccaccccaggtgcccagatggtccccaattagagcagaggaaaggacaagtccagatagctatgtagagcccactgcaatgaagccagctgaa

SEQ ID NO: 28 - DNA, 137 bp, Artificial Sequence
  ssODNs PRKDC Cas9n
gcgaaggcccaagcgcatcatcatccgtggccatgacgagagggaacaccctttcctggtgagaggtggcgaggacctgcggcaggaccagcgcgtggagcagctcttccaggtcatgaatgggatcctggcccaag

SEQ ID NO: 29 - DNA, 103 bp, Artificial Sequence
  ssODNs POLQ Cas9n
tgagtcaatgagcatgtactagaatgtaacagggcacatggattccattgttatcccatttcaactaagtcctgctgcagaatcattctggcttcttccacta

SEQ ID NO: 30 - DNA, 20 bp, Artificial Sequence
  Primer SCAP forward
aagcgttcccagtcattctg

SEQ ID NO: 31 - DNA, 20 bp, Artificial Sequence
  Primer SCAP reverse
ctttggcgataccagagagc

SEQ ID NO: 32 - DNA, 23 bp, Artificial Sequence
  Primer LYPLA1 forward
aaaaactgctgtacacaaaagca

SEQ ID NO: 33 - DNA, 25 bp, Artificial Sequence
  Primer LYPLA1 reverse
tgtgtaggtctcaagcaattatctg

SEQ ID NO: 34 - DNA, 20 bp, Artificial Sequence
  Primer SSH2 forward
tcaggactccttcctgctgt

SEQ ID NO: 35 - DNA, 20 bp, Artificial Sequence
  Primer SSH2 reverse
gcaccaaaagggaaaagtga

SEQ ID NO: 36 - DNA, 20 bp, Artificial Sequence
  Primer VCAN forward
ggcaggattccacgatagca

SEQ ID NO: 37 - DNA, 20 bp, Artificial Sequence
  Primer VCAN reverse
cgtgccttccactgactctt

SEQ ID NO: 38 - DNA, 20 bp, Artificial Sequence
  Primer CSGALNACT1 forward
gatgctgtcagtggtcagga

SEQ ID NO: 39 - DNA, 21 bp, Artificial Sequence
  Primer CSGALNACT1 reverse
tcttaccgtgcaaagaaggag

SEQ ID NO: 40 - DNA, 20 bp, Artificial Sequence
  Primer ITGB4 forward
ccatagagtcccaggatgga

SEQ ID NO: 41 - DNA, 20 bp, Artificial Sequence
  Primer ITGB4 reverse
gtgctcacccactaggaagg

SEQ ID NO: 42 - DNA, 20 bp, Artificial Sequence
  Primer FRMD7 forward
tgctcctaccgctagtcctg

SEQ ID NO: 43 - DNA, 20 bp, Artificial Sequence
  FRMD7 reverse
ggtattatgcctccccaggt

SEQ ID NO: 44 - DNA, 20 bp, Artificial Sequence
  Primer PRKDC forward
ctagcctgtgccctgagatg

SEQ ID NO: 45 - DNA, 21 bp, Artificial Sequence
  Primer PRKDC reverse
gcacaacgctataggtcctca

SEQ ID NO: 46 - DNA, 20 bp, Artificial Sequence
  Primer POLQ forward
ttccaaaatcctcatgcaca

SEQ ID NO: 47 - DNA, 21 bp, Artificial Sequence
  Primer POLQ reverse
tgctgatcagttttgctcctt

SEQ ID NO: 48 - DNA, 33 bp, Artificial Sequence
  Primer Illumina adapter forward 5'
acactctttccctacacgacgctcttccgatct

SEQ ID NO: 49 - DNA, 34 bp, Artificial Sequence
  Primer Illumina adapter reverse 5'
gtgactggagttcagacgtgtgctcttccgatct

SEQ ID NO: 50 - DNA, 20 bp, Artificial Sequence
  VCAN gRNA1
gtttactgttgcctgatcat

SEQ ID NO: 51 - DNA, 20 bp, Artificial Sequence
  VCAN gRNA2
ccctgtggaatttaatactg

SEQ ID NO: 52 - DNA, 101 bp, Artificial Sequence; identical to SEQ ID NO: 23
  VCAN donor ssDNA

SEQ ID NO: 53 - DNA, 20 bp, Artificial Sequence
  NFASC gRNA1
tgtagtagttgtggcgacgg

SEQ ID NO: 54 - DNA, 20 bp, Artificial Sequence
  NFASC gRNA2
tgctgccgccaccaccacca

SEQ ID NO: 55 - DNA, 107 bp, Artificial Sequence
  NFASC donor ssDNA
ggattcgtgtatcttagtcccggaggtggtggtgggaggactctccgtggttgtggtggtggcagcagtggttgtagtagttgtggcgacggtggtggtggtggcga

SEQ ID NO: 56 - DNA, 20 bp, Artificial Sequence
  PolQ gRNA1
tagttgaaatgggagtgcaa

SEQ ID NO: 57 - DNA, 20 bp, Artificial Sequence
  PolQ gRNA2 (coding strand)
gtcctgctgcagaatcattc

SEQ ID NO: 58 - DNA, 103 bp, PolQ KO donor ssDNA; identical to SEQ ID NO: 29

SEQ ID NO: 59 - DNA, 19 bp, Artificial Sequence
  PolQ siRNA SMART pool
caacaacccttatcgtaaa

SEQ ID NO: 60 - DNA, 19 bp, Artificial Sequence
  PolQ siRNA SMART pool
cgactaagatagatcattt

SEQ ID NO: 61 - DNA, 19 bp, Artificial Sequence
  PolQ siRNA SMART pool
acacagtaggcgagagtat

SEQ ID NO: 62 - DNA, 19 bp, Artificial Sequence
  PolQ siRNA SMART pool
ccttaagactgtaggtact

SEQ ID NO: 63 - DNA, 27 bp, Artificial Sequence
  PolQ siRNA aa765
ttggaaaatactgtaatcatccctgca